European Patent Application EP 4 736 885 A1, published May 6, 2026. Title: 抗体-药物偶联物及其用途. Applicant: 石药集团巨石生物制药有限公司. The sequence listing filed with the application follows.

SEQUENCE LISTING (25 sequences)

SEQ ID NO: 1 - protein, 5 aa, Synthetic construct
DYFMN

SEQ ID NO: 2 - protein, 17 aa, Synthetic construct
DVNPKTGSPSYNQKFKG

SEQ ID NO: 3 - protein, 10 aa, Synthetic construct
RYGFLYSMDY

SEQ ID NO: 4 - protein, 11 aa, Synthetic construct
RASQDISNYLN

SEQ ID NO: 5 - protein, 7 aa, Synthetic construct
YTSRLHS

SEQ ID NO: 6 - protein, 9 aa, Synthetic construct
QQGNTHPFT

SEQ ID NO: 7 - protein, 119 aa, Synthetic construct
QVQLVQSGAEVKKPGASVKVSCKASGYTFTDYFMNWVRQAPGQGLEWMGDVNPKTGSPSYNQKFKGRVTMTRDTSTSTVYMELSSLRSEDTAVYYCARRYGFLYSMDYWGQGTSVTVSS

SEQ ID NO: 8 - protein, 107 aa, Synthetic construct
DIQMTQSPSSLSASVGDRVTITCRASQDISNYLNWYQQKPGKAVKVLIYYTSRLHSGVPSRFSGSGSGTDFTFTISSLQPEDIATYYCQQGNTHPFTFGGGTKVEIK

SEQ ID NO: 9 - protein, 449 aa, Synthetic construct
QVQLVQSGAEVKKPGASVKVSCKASGYTFTDYFMNWVRQAPGQGLEWMGDVNPKTGSPSYNQKFKGRVTMTRDTSTSTVYMELSSLRSEDTAVYYCARRYGFLYSMDYWGQGTSVTVSSASTKGPSVFPLAPSSKSTSGGTAALGCLVKDYFPEPVTVSWNSGALTSGVHTFPAVLQSSGLYSLSSVVTVPSSSLGTQTYICNVNHKPSNTKVDKRVEPKSCDKTHTCPPCPAPEAAGGPSVFLFPPKPKDTLMISRTPEVTCVVVDVSHEDPEVKFNWYVDGVEVHNAKTKPREEQYNSTYRVVSVLTVLHQDWLNGKEYKCKVSNKALAASIEKTISKAKGQPREPQVYTLPPSREEMTKNQVSLTCLVKGFYPSDIAVEWESNGQPENNYKTTPPVLDSDGSFFLYSKLTVDKSRWQQGNVFSCSVMHEALHNHYTQKSLSLSPGK

SEQ ID NO: 10 - protein, 449 aa, Synthetic construct
QVQLVQSGAEVKKPGASVKVSCKASGYTFTDYFMNWVRQAPGQGLEWMGDVNPKTGSPSYNQKFKGRVTMTRDTSTSTVYMELSSLRSEDTAVYYCARRYGFLYSMDYWGQGTSVTVSSASTKGPSVFPLAPSSKSTSGGTAALGCLVKDYFPEPVTVSWNSGALTSGVHTFPAVLQSSGLYSLSSVVTVPSSSLGTQTYICNVNHKPSNTKVDKRVEPKSCDKTHTSPPCPAPEAAGGPSVFLFPPKPKDTLMISRTPEVTCVVVDVSHEDPEVKFNWYVDGVEVHNAKTKPREEQYNSTYRVVSVLTVLHQDWLNGKEYKCKVSNKALAASIEKTISKAKGQPREPQVYTLPPSREEMTKNQVSLTCLVKGFYPSDIAVEWESNGQPENNYKTTPPVLDSDGSFFLYSKLTVDKSRWQQGNVFSCSVMHEALHNHYTQKSLSLSPGK

SEQ ID NO: 11 - protein, 214 aa, Synthetic construct
DIQMTQSPSSLSASVGDRVTITCRASQDISNYLNWYQQKPGKAVKVLIYYTSRLHSGVPSRFSGSGSGTDFTFTISSLQPEDIATYYCQQGNTHPFTFGGGTKVEIKRTVAAPSVFIFPPSDEQLKSGTASVVCLLNNFYPREAKVQWKVDNALQSGNSQESVTEQDSKDSTYSLSSTLTLSKADYEKHKVYACEVTHQGLSSPVTKSFNRGEC

SEQ ID NO: 12 - protein, 450 aa, Synthetic construct
EVQLVESGGGLVQPGGSLRLSCAASGFNIKDTYIHWVRQAPGKGLEWVARIYPTNGYTRYADSVKGRFTISADTSKNTAYLQMNSLRAEDTAVYYCSRWGGDGFYAMDYWGQGTLVTVSSASTKGPSVFPLAPSSKSTSGGTAALGCLVKDYFPEPVTVSWNSGALTSGVHTFPAVLQSSGLYSLSSVVTVPSSSLGTQTYICNVNHKPSNTKVDKKVEPKSCDKTHTCPPCPAPELLGGPSVFLFPPKPKDTLMISRTPEVTCVVVDVSHEDPEVKFNWYVDGVEVHNAKTKPREEQYNSTYRVVSVLTVLHQDWLNGKEYKCKVSNKALPAPIEKTISKAKGQPREPQVYTLPPSREEMTKNQVSLTCLVKGFYPSDIAVEWESNGQPENNYKTTPPVLDSDGSFFLYSKLTVDKSRWQQGNVFSCSVMHEALHNHYTQKSLSLSPGK

SEQ ID NO: 13 - protein, 214 aa, Synthetic construct
DIQMTQSPSSLSASVGDRVTITCRASQDVNTAVAWYQQKPGKAPKLLIYSASFLYSGVPSRFSGSRSGTDFTLTISSLQPEDFATYYCQQHYTTPPTFGQGTKVEIKRTVAAPSVFIFPPSDEQLKSGTASVVCLLNNFYPREAKVQWKVDNALQSGNSQESVTEQDSKDSTYSLSSTLTLSKADYEKHKVYACEVTHQGLSSPVTKSFNRGEC

SEQ ID NO: 14 - protein, 451 aa, Synthetic construct
QVQLQQSGSELKKPGASVKVSCKASGYTFTNYGMNWVKQAPGQGLKWMGWINTYTGEPTYTDDFKGRFAFSLDTSVSTAYLQISSLKADDTAVYFCARGGFGSSYWYFDVWGQGSLVTVSSASTKGPSVFPLAPSSKSTSGGTAALGCLVKDYFPEPVTVSWNSGALTSGVHTFPAVLQSSGLYSLSSVVTVPSSSLGTQTYICNVNHKPSNTKVDKRVEPKSCDKTHTCPPCPAPELLGGPSVFLFPPKPKDTLMISRTPEVTCVVVDVSHEDPEVKFNWYVDGVEVHNAKTKPREEQYNSTYRVVSVLTVLHQDWLNGKEYKCKVSNKALPAPIEKTISKAKGQPREPQVYTLPPSREEMTKNQVSLTCLVKGFYPSDIAVEWESNGQPENNYKTTPPVLDSDGSFFLYSKLTVDKSRWQQGNVFSCSVMHEALHNHYTQKSLSLSPGK

SEQ ID NO: 15 - protein, 214 aa, Synthetic construct
DIQLTQSPSSLSASVGDRVSITCKASQDVSIAVAWYQQKPGKAPKLLIYSASYRYTGVPDRFSGSGSGTDFTLTISSLQPEDFAVYYCQQHYITPLTFGAGTKVEIKRTVAAPSVFIFPPSDEQLKSGTASVVCLLNNFYPREAKVQWKVDNALQSGNSQESVTEQDSKDSTYSLSSTLTLSKADYEKHKVYACEVTHQGLSSPVTKSFNRGEC

SEQ ID NO: 16 - protein, 450 aa, Synthetic construct
QLQLQESGPGLVKPSETLSLTCTVSGGSIKSGSYYWGWIRQPPGKGLEWIGNIYYSGSTYYNPSLRSRVTISVDTSKNQFSLKLSSVTAADTAVYYCAREGSYPNQFDPWGQGTLVTVSSASTKGPSVFPLAPSSKSTSGGTAALGCLVKDYFPEPVTVSWNSGALTSGVHTFPAVLQSSGLYSLSSVVTVPSSSLGTQTYICNVNHKPSNTKVDKKVEPKSCDKTHTCPPCPAPELLGGPSVFLFPPKPKDTLMISRTPEVTCVVVDVSHEDPEVKFNWYVDGVEVHNAKTKPREEQYNSTYRVVSVLTVLHQDWLNGKEYKCKVSNKALPAPIEKTISKAKGQPREPQVYTLPPSRDELTKNQVSLTCLVKGFYPSDIAVEWESNGQPENNYKTTPPVLDSDGSFFLYSKLTVDKSRWQQGNVFSCSVMHEALHNHYTQKSLSLSPGK

SEQ ID NO: 17 - protein, 214 aa, Synthetic construct
EIVMTQSPATLSVSPGERATLSCRASQSVSSNLAWYQQKPGQAPRLLIYGASTRATGIPARFSGSGSGTEFTLTISSLQSEDFAVYYCQQYHSFPFTFGGGTKVEIKRTVAAPSVFIFPPSDEQLKSGTASVVCLLNNFYPREAKVQWKVDNALQSGNSQESVTEQDSKDSTYSLSSTLTLSKADYEKHKVYACEVTHQGLSSPVTKSFNRGEC

SEQ ID NO: 18 - protein, 448 aa, Synthetic construct
EVQLLESGGGLVQPGGSLRLSCAASGFTFSNYAMSWVRQAPGKGLEWVSSISGSGDYTYYTDSVKGRFTISRDNSKNTLYLQMNSLRAEDTAVYYCARSPWGYYLDSWGQGTLVTVSSASTKGPSVFPLAPSSKSTSGGTAALGCLVKDYFPEPVTVSWNSGALTSGVHTFPAVLQSSGLYSLSSVVTVPSSSLGTQTYICNVNHKPSNTKVDKRVEPKSCDKTHTCPPCPAPELLGGPSVFLFPPKPKDTLMISRTPEVTCVVVDVSHEDPEVKFNWYVDGVEVHNAKTKPREEQYNSTYRVVSVLTVLHQDWLNGKEYKCKVSNKALPAPIEKTISKAKGQPREPQVYTLPPSREEMTKNQVSLTCLVKGFYPSDIAVEWESNGQPENNYKTTPPVLDSDGSFFLYSKLTVDKSRWQQGNVFSCSVMHEALHNHYTQKSLSLSPGK

SEQ ID NO: 19 - protein, 214 aa, Synthetic construct
DIQMTQSPPSLSASAGDRVTITCRASQGISSRLAWYQQKPEKAPKSLIYAASSLQSGVPSRFSGSGSGTDFTLTISSLQPEDFATYYCQQYNSYPYTFGQGTKLEIKRTVAAPSVFIFPPSDEQLKSGTASVVCLLNNFYPREAKVQWKVDNALQSGNSQESVTEQDSKDSTYSLSSTLTLSKADYEKHKVYACEVTHQGLSSPVTKSFNRGEC

SEQ ID NO: 20 - protein, 445 aa, Synthetic construct
EVQLLESGGGLVQPGGSLRLSCAASGFTFSSFSMSWVRQAPGKGLEWVSSISGSSGTTYYADSVKGRFTISRDNSKNTLYLQMNSLRAEDTAVYYCARPFPYFDYWGQGTLVTVSSASTKGPSVFPLAPSSKSTSGGTAALGCLVKDYFPEPVTVSWNSGALTSGVHTFPAVLQSSGLYSLSSVVTVPSSSLGTQTYICNVNHKPSNTKVDKKVEPKSCDKTHTCPPCPAPELLGGPSVFLFPPKPKDTLMISRTPEVTCVVVDVSHEDPEVKFNWYVDGVEVHNAKTKPREEQYNSTYRVVSVLTVLHQDWLNGKEYKCKVSNKALPAPIEKTISKAKGQPREPQVYTLPPSREEMTKNQVSLTCLVKGFYPSDIAVEWESNGQPENNYKTTPPVLDSDGSFFLYSKLTVDKSRWQQGNVFSCSVMHEALHNHYTQKSLSLSPG

SEQ ID NO: 21 - protein, 215 aa, Synthetic construct
EIVLTQSPGTLSLSPGERATLSCRASQSVSSSFLAWYQQKPGQAPRLLIYYASSRATGIPDRFSGSGSGTDFTLTISRLEPEDFAVYYCQQTGRIPPTFGQGTKVEIKRTVAAPSVFIFPPSDEQLKSGTASVVCLLNNFYPREAKVQWKVDNALQSGNSQESVTEQDSKDSTYSLSSTLTLSKADYEKHKVYACEVTHQGLSSPVTKSFNRGEC

SEQ ID NO: 22 - protein, 448 aa, Synthetic construct
QVQLQQPGAELVRPGASVKLSCKASGYTFTSYWINWVKQRPGQGLEWIGNIYPSDSYTNYNQKFKDKATLTVDKSSSTAYMQLSSPTSEDSAVYYCTRSWRGNSFDYWGQGTTLTVSSASTKGPSVFPLAPSSKSTSGGTAALGCLVKDYFPEPVTVSWNSGALTSGVHTFPAVLQSSGLYSLSSVVTVPSSSLGTQTYICNVNHKPSNTKVDKRVEPKSCDKTHTCPPCPAPELLGGPSVFLFPPKPKDTLMISRTPEVTCVVVDVSHEDPEVKFNWYVDGVEVHNAKTKPREEQYNSTYRVVSVLTVLHQDWLNGKEYKCKVSNKALPAPIEKTISKAKGQPREPQVYTLPPSREEMTKNQVSLTCLVKGFYPSDIAVEWESNGQPENNYKTTPPVLDSDGSFFLYSKLTVDKSRWQQGNVFSCSVMHEALHNHYTQKSLSLSPGK

SEQ ID NO: 23 - protein, 220 aa, Synthetic construct
DIVMTQSPSSLTVTAGEKVTMSCKSSQSLLNSGNQKNYLTWYQQKPGQPPKLLIYWASTRESGVPDRFTGSGSGTDFTLTISSVQAEDLAVYYCQNDYSYPFTFGSGTKLEIKRTVAAPSVFIFPPSDEQLKSGTASVVCLLNNFYPREAKVQWKVDNALQSGNSQESVTEQDSKDSTYSLSSTLTLSKADYEKHKVYACEVTHQGLSSPVTKSFNRGEC

SEQ ID NO: 24 - protein, 452 aa, Synthetic construct
QVQLVQSGAEVKKPGSSVKVSCKASGYTFTNYVMHWVRQAPGQGLEWMGYINPYNDDVKYNEKFKGRVTITADESTSTAYMELSSLRSEDTAVYYCARWGYYGSPLYYFDYWGQGTLVTVSSASTKGPSVFPLAPSSKSTSGGTAALGCLVKDYFPEPVTVSWNSGALTSGVHTFPAVLQSSGLYSLSSVVTVPSSSLGTQTYICNVNHKPSNTKVDKRVEPKSCDKTHTCPPCPAPELLGGPSVFLFPPKPKDTLMISRTPEVTCVVVDVSHEDPEVKFNWYVDGVEVHNAKTKPREEQYNSTYRVVSVLTVLHQDWLNGKEYKCKVSNKALPAPIEKTISKAKGQPREPQVYTLPPSREEMTKNQVSLTCLVKGFYPSDIAVEWESNGQPENNYKTTPPVLDSDGSFFLYSKLTVDKSRWQQGNVFSCSVMHEALHNHYTQKSLSLSPGK

SEQ ID NO: 25 - protein, 213 aa, Synthetic construct
EIVLTQSPATLSLSPGERATLSCRASSRLIYMHWYQQKPGQAPRPLIYATSNLASGIPARFSGSGSGTDFTLTISSLEPEDFAVYYCQQWNSNPPTFGQGTKVEIKRTVAAPSVFIFPPSDEQLKSGTASVVCLLNNFYPREAKVQWKVDNALQSGNSQESVTEQDSKDSTYSLSSTLTLSKADYEKHKVYACEVTHQGLSSPVTKSFNRGEC